European Patent Specification EP 3 497 117 B1, published January 24, 2024. Title: Alkaline stable Immunoglobulin-binding proteins. Applicant: Navigo Proteins GmbH. The sequence listing filed with the application follows.

SEQUENCE LISTING (55 sequences)

SEQ ID NO: 1 - protein, 58 aa, Artificial Sequence
  generic sequence 1
  variant (1)..(1): may be replaced by V, N, Q, or P
  variant (2)..(2): may be replaced by D or Q
  variant (3)..(3): may be replaced by N or S
  variant (4)..(4): may be replaced by  N
  variant (5)..(5): may be replaced by F
  variant (6)..(6): may be replaced by N, A, or S
  variant (7)..(7): may be replaced by E
  variant (8)..(8): may be replaced by E or A
  variant (11)..(11): may be replaced by N
  variant (15)..(15): may be replaced by Q
  variant (16)..(16): may be replaced by V
  variant (18)..(18): may be replaced by N
  variant (19)..(19): may be replaced by M
  variant (21)..(21): may be replaced by S or D
  variant (23)..(23): may be replaced by N
  variant (24)..(24): may be replaced by A
  variant (25)..(25): may be replaced by E
  variant (28)..(28): may be replaced by S or A
  variant (29)..(29): may be replaced by G
  variant (40)..(40): may be replaced by Q or T
  variant (42)..(42): may be replaced by A or T
  variant (43)..(43): may be replaced by N or S
  variant (44)..(44): may be replaced by V or L
  variant (46)..(46): may be replaced by A
  variant (49)..(49): may be replaced by Q
  variant (52)..(52): may be replaced by D or S
  variant (53)..(53): may be replaced by E
  variant (54)..(54): may be replaced by S
  variant (58)..(58): may be replaced by K
AAAKHDKDQQSAFYEILHLPNLTEDQRNAFIQSLKDDPSVSKEILGEAKKLNDAQAPP

SEQ ID NO: 2 - protein, 58 aa, Artificial Sequence; identical to SEQ ID NO: 1
  Generic sequence 2
  variant (1)..(1): may be replaced by N or P
  variant (5)..(5): may be replaced by F
  variant (7)..(7): may be replaced by E
  variant (8)..(8): may be replaced by E or A
  variant (11)..(11): may be replaced by N
  variant (25)..(25): may be replaced by E
  variant (28)..(28): may be replaced by S
  variant (44)..(44): may be replaced by V
  variant (46)..(46): may be replaced by A
  variant (49)..(49): may be replaced by Q
  variant (54)..(54): may be replaced by S
  variant (58)..(58): may be replaced by K

SEQ ID NO: 3 - protein, 58 aa, Artificial Sequence; identical to SEQ ID NO: 1
  parental protein IB14 1A/28N (IB14a)

SEQ ID NO: 4 - protein, 58 aa, Artificial Sequence
  parental protein IB27 1A
AAAKFDEAQQSAFYEILHLPNLTEEQRNAFIQSLKDDPSVSKEVLGEAQKLNDSQAPK

SEQ ID NO: 5 - protein, 58 aa, Artificial Sequence
  domain C
ADNKFNKEQQNAFYEILHLPNLTEEQRNGFIQSLKDDPSVSKEILAEAKKLNDAQAPK

SEQ ID NO: 6 - protein, 58 aa, Artificial Sequence [sequence omitted]

SEQ ID NO: 7 - protein, 58 aa, Artificial Sequence [sequence omitted]

SEQ ID NO: 8 - protein, 58 aa, Artificial Sequence [sequence omitted]

SEQ ID NO: 9 - protein, 58 aa, Artificial Sequence
  IB14 1I
IAAKHDKDQQSAFYEILHLPNLTEDQRSAFIQSLKDDPSVSKEILGEAKKLNDAQAPP

SEQ ID NO: 10 - protein, 58 aa, Artificial Sequence
  IB14 1A/28S (IB14b)
AAAKHDKDQQSAFYEILHLPNLTEDQRSAFIQSLKDDPSVSKEILGEAKKLNDAQAPP

SEQ ID NO: 11 - protein, 58 aa, Artificial Sequence
  IB14 11A
PAAKHDKDQQAAFYEILHLPNLTEDQRSAFIQSLKDDPSVSKEILGEAKKLNDAQAPP

SEQ ID NO: 12 - protein, 58 aa, Artificial Sequence
  IB14 11E
PAAKHDKDQQEAFYEILHLPNLTEDQRSAFIQSLKDDPSVSKEILGEAKKLNDAQAPP

SEQ ID NO: 13 - protein, 58 aa, Artificial Sequence
  IB14 11I
PAAKHDKDQQIAFYEILHLPNLTEDQRSAFIQSLKDDPSVSKEILGEAKKLNDAQAPP

SEQ ID NO: 14 - protein, 58 aa, Artificial Sequence
  IB14 1P 28S (IB14d)
PAAKHDKDQQSAFYEILHLPNLTEDQRSAFIQSLKDDPSVSKEILGEAKKLNDAQAPP

SEQ ID NO: 15 - protein, 58 aa, Artificial Sequence
  IB14 35R
PAAKHDKDQQSAFYEILHLPNLTEDQRSAFIQSLRDDPSVSKEILGEAKKLNDAQAPP

SEQ ID NO: 16 - protein, 58 aa, Artificial Sequence
  IB14 35I
PAAKHDKDQQSAFYEILHLPNLTEDQRSAFIQSLIDDPSVSKEILGEAKKLNDAQAPP

SEQ ID NO: 17 - protein, 58 aa, Artificial Sequence
  IB14 42L
PAAKHDKDQQSAFYEILHLPNLTEDQRSAFIQSLKDDPSVSLEILGEAKKLNDAQAPP

SEQ ID NO: 18 - protein, 58 aa, Artificial Sequence
  alkaline stable Ig binding domain cs14-1 (IB14 1I/11A/35R )
IAAKHDKDQQAAFYEILHLPNLTEDQRSAFIQSLRDDPSVSKEILGEAKKLNDAQAPP

SEQ ID NO: 19 - protein, 58 aa, Artificial Sequence
  alkaline stable Ig binding domain cs14-2 (IB14 1I/11A/35R/42L)
IAAKHDKDQQAAFYEILHLPNLTEDQRSAFIQSLRDDPSVSLEILGEAKKLNDAQAPP

SEQ ID NO: 20 - protein, 58 aa, Artificial Sequence
  alkaline stable Ig binding domain cs14-3  1I/11A/28N/35R/42L
IAAKHDKDQQAAFYEILHLPNLTEDQRNAFIQSLRDDPSVSLEILGEAKKLNDAQAPP

SEQ ID NO: 21 - protein, 58 aa, Artificial Sequence
  IB14 1P/28N (IB14c)
PAAKHDKDQQSAFYEILHLPNLTEDQRNAFIQSLKDDPSVSKEILGEAKKLNDAQAPP

SEQ ID NO: 22 - protein, 58 aa, Artificial Sequence
  IB27 1N
NAAKFDEAQQSAFYEILHLPNLTEEQRNAFIQSLKDDPSVSKEVLGEAQKLNDSQAPK

SEQ ID NO: 23 - protein, 53 aa, Artificial Sequence
  cs27 delNC
KFDEAQQAAFYEILHLPNLTEEQRNAFIQSLRDDPSVSLEVLGEAQKLNDSQA

SEQ ID NO: 24 - protein, 55 aa, Artificial Sequence
  cs27 delN
AFDEAQQAAFYEILHLPNLTEEQRNAFIQSLRDDPSVSLEVLGEAQKLNDSQAPK

SEQ ID NO: 25 - protein, 58 aa, Artificial Sequence
  parental protein IB25 1A
AAAKHDKDQQSAFYEILHLPNLTEDQRNAFIQSLKDDPSVSKEILAEAKKLNDAQAPK

SEQ ID NO: 26 - protein, 58 aa, Artificial Sequence
  alkaline stable Ig binding domain cs25 (IB25 1I/11A/35R/42L)
IAAKHDKDQQAAFYEILHLPNLTEDQRNAFIQSLRDDPSVSLEILAEAKKLNDAQAPK

SEQ ID NO: 27 - protein, 318 aa, Artificial Sequence
  cs17 delNC hexamer
KFDEAQQAAFYEILHLPNLTEEQRNAFIQSLRDDPSVSLEVLGEAQKLNDSQAKFDEAQQAAFYEILHLPNLTEEQRNAFIQSLRDDPSVSLEVLGEAQKLNDSQAKFDEAQQAAFYEILHLPNLTEEQRNAFIQSLRDDPSVSLEVLGEAQKLNDSQAKFDEAQQAAFYEILHLPNLTEEQRNAFIQSLRDDPSVSLEVLGEAQKLNDSQAKFDEAQQAAFYEILHLPNLTEEQRNAFIQSLRDDPSVSLEVLGEAQKLNDSQAKFDEAQQAAFYEILHLPNLTEEQRNAFIQSLRDDPSVSLEVLGEAQKLNDSQA

SEQ ID NO: 28 - protein, 290 aa, Artificial Sequence
  cs27 pentamer
IAAKFDEAQQAAFYEILHLPNLTEEQRNAFIQSLRDDPSVSLEVLGEAQKLNDSQAPKIAAKFDEAQQAAFYEILHLPNLTEEQRNAFIQSLRDDPSVSLEVLGEAQKLNDSQAPKIAAKFDEAQQAAFYEILHLPNLTEEQRNAFIQSLRDDPSVSLEVLGEAQKLNDSQAPKIAAKFDEAQQAAFYEILHLPNLTEEQRNAFIQSLRDDPSVSLEVLGEAQKLNDSQAPKIAAKFDEAQQAAFYEILHLPNLTEEQRNAFIQSLRDDPSVSLEVLGEAQKLNDSQAPK

SEQ ID NO: 29 - protein, 58 aa, Artificial Sequence
  alkaline stable Ig binding domain cs27-1 (IB27 1I/11A/35R)
IAAKFDEAQQAAFYEILHLPNLTEEQRNAFIQSLRDDPSVSKEVLGEAQKLNDSQAPK

SEQ ID NO: 30 - protein, 58 aa, Artificial Sequence
  alkaline stable Ig binding domain cs27-2 (IB27 I/11A/35R/42L)
IAAKFDEAQQAAFYEILHLPNLTEEQRNAFIQSLRDDPSVSLEVLGEAQKLNDSQAPK

SEQ ID NO: 31 - protein, 58 aa, Artificial Sequence
  alkaline stable Ig binding domain C 1I/11A/35R
IDNKFNKEQQAAFYEILHLPNLTEEQRNGFIQSLRDDPSVSKEILAEAKKLNDAQAPK

SEQ ID NO: 32 - protein, 58 aa, Artificial Sequence
  alkaline stable Ig binding domain C 1I/11A/35R/42L
IDNKFNKEQQAAFYEILHLPNLTEEQRNGFIQSLRDDPSVSLEILAEAKKLNDAQAPK

SEQ ID NO: 33 - protein, 58 aa, Artificial Sequence
  alkaline stable Ig binding domain B 1I/11A/35R
IDNKFNKEQQAAFYEILHLPNLNEEQRNGFIQSLRDDPSQSANLLAEAKKLNDAQAPK

SEQ ID NO: 34 - protein, 58 aa, Artificial Sequence
  alkaline stable Ig binding domain B 1I/11A/35R/42L
IDNKFNKEQQAAFYEILHLPNLNEEQRNGFIQSLRDDPSQSLNLLAEAKKLNDAQAPK

SEQ ID NO: 35 - protein, 58 aa, Artificial Sequence
  alkaline stable Ig binding domain  Z 1I/11A/35R
IDNKFNKEQQAAFYEILHLPNLNEEQRNAFIQSLRDDPSQSANLLAEAKKLNDAQAPK

SEQ ID NO: 36 - protein, 58 aa, Artificial Sequence
  alkaline stable Ig binding domain  Z 1I/11A/35R/42L
IDNKFNKEQQAAFYEILHLPNLNEEQRNAFIQSLRDDPSQSLNLLAEAKKLNDAQAPK

SEQ ID NO: 37 - protein, 58 aa, Artificial Sequence
  alkaline stable Ig binding domain domain Z/2 1I/11A/35R
IDAKFDKEQQAAFYEILHLPNLTEEQRNAFIQSLRDDPSQSLALLAEAKKLNDAQAPK

SEQ ID NO: 38 - protein, 58 aa, Artificial Sequence
  alkaline stable Ig binding domain Z/2 1I/11A/35R/42L
IDAKFDKEQQAAFYEILHLPNLTEEQRNAFIQSLRDDPSQSLNLLAEAKKLNDAQAPK

SEQ ID NO: 39 - protein, 79 aa, Artificial Sequence
  alkaline stable Ig binding domain cs14-3 with coupling sequence and strep tag
IAAKHDKDQQAAFYEILHLPNLTEDQRNAFIQSLRDDPSVSLEILGEAKKLNDAQAPPASPAPSAPSACASWSHPQFEK

SEQ ID NO: 40 - protein, 79 aa, Artificial Sequence
  alkaline stable Ig binding domain cs27-2 with coupling sequence and strep tag
IAAKFDEAQQAAFYEILHLPNLTEEQRNAFIQSLRDDPSVSLEVLGEAQKLNDSQAPKASPAPSAPSACASWSHPQFEK

SEQ ID NO: 41 - protein, 13 aa, Artificial Sequence
  coupling sequence
ASPAPSAPSACAS

SEQ ID NO: 42 - protein, 58 aa, Artificial Sequence
  alkaline stable Ig binding domain cs74h1
IAAKFDEAQQAAFYEILHLPNLTEDQRNAFIQSLRDDPSVSLEILGEAKKLNDAQAPP

SEQ ID NO: 43 - protein, 58 aa, Artificial Sequence
  alkaline stable Ig binding domain cs74h2
IAAKFDEAQQAAFYEILHLPNLTEEQRNAFIQSLRDDPSVSLEILGEAKKLNDAQAPP

SEQ ID NO: 44 - protein, 58 aa, Artificial Sequence
  alkaline stable Ig binding domain cs47h3
IAAKHDKDQQAAFYEILHLPNLTEDQRNAFIQSLRDDPSVSLEVLGEAQKLNDSQAPK

SEQ ID NO: 45 - protein, 58 aa, Artificial Sequence
  alkaline stable Ig binding domain cs47h4
IAAKHDKDQQAAFYEILHLPNLTEEQRNAFIQSLRDDPSVSLEVLGEAQKLNDSQAPK

SEQ ID NO: 46 - protein, 8 aa, Artificial Sequence
  StrepTag
WSHPQFEK

SEQ ID NO: 47 - protein, 58 aa, Artificial Sequence
  parental protein IB74h1
AAAKFDEAQQSAFYEILHLPNLTEDQRNAFIQSLKDDPSVSKEILGEAKKLNDAQAPP

SEQ ID NO: 48 - protein, 58 aa, Artificial Sequence
  parental protein IB74h2
AAAKFDEAQQSAFYEILHLPNLTEEQRNAFIQSLKDDPSVSKEILGEAKKLNDAQAPP

SEQ ID NO: 49 - protein, 58 aa, Artificial Sequence
  parental protein IB47h3
AAAKHDKDQQSAFYEILHLPNLTEDQRNAFIQSLKDDPSVSKEVLGEAQKLNDSQAPK

SEQ ID NO: 50 - protein, 58 aa, Artificial Sequence
  parental protein IB47h4
AAAKHDKDQQSAFYEILHLPNLTEEQRNAFIQSLKDDPSVSKEVLGEAQKLNDSQAPK

SEQ ID NO: 51 - protein, 58 aa, Artificial Sequence; identical to SEQ ID NO: 1
  generic sequence including IB14 and IB27
  variant (1)..(1): may be replaced by N or P
  variant (5)..(5): may be replaced by F
  variant (7)..(7): may be replaced by E
  variant (8)..(8): may be replaced by A
  variant (25)..(25): may be replaced by E
  variant (28)..(28): may be replaced by S
  variant (44)..(44): may be replaced by V
  variant (49)..(49): may be replaced by Q
  variant (54)..(54): may be replaced by S
  variant (58)..(58): may be replaced by K

SEQ ID NO: 52 - protein, 58 aa, Artificial Sequence
  Generic sequence of preferred alkaline stable artifical IgG binding proteins
  variant (5)..(5): may be replaced by F
  variant (7)..(7): may be replaced by E
  variant (8)..(8): may be replaced by A or E
  variant (25)..(25): may be replaced by E
  variant (28)..(28): may be replaced by S
  variant (42)..(42): may be replaced by L
  variant (44)..(44): may be replaced by V
  variant (46)..(46): may be replaced by A
  variant (49)..(49): may be replaced by Q
  variant (54)..(54): may be replaced by S
  variant (58)..(58): may be replaced by K
IAAKHDKDQQAAFYEILHLPNLTEDQRNAFIQSLRDDPSVSKEILGEAKKLNDAQAPP

SEQ ID NO: 53 - protein, 58 aa, Artificial Sequence
  cs27 46C
IAAKFDEAQQAAFYEILHLPNLTEEQRNAFIQSLRDDPSVSLEVLCEAQKLNDSQAPK

SEQ ID NO: 54 - protein, 58 aa, Artificial Sequence
  cs14 43C
IAAKHDKDQQAAFYEILHLPNLTEDQRNAFIQSLRDDPSVSLCILGEAKKLNDAQAPP

SEQ ID NO: 55 - protein, 174 aa, Artificial Sequence
  cs27 tetramer
IAAKFDEAQQAAFYEILHLPNLTEEQRNAFIQSLRDDPSVSLEVLGEAQKLNDSQAPKIAAKFDEAQQAAFYEILHLPNLTEEQRNAFIQSLRDDPSVSLEVLGEAQKLNDSQAPKIAAKFDEAQQAAFYEILHLPNLTEEQRNAFIQSLRDDPSVSLEVLGEAQKLNDSQAPK